European Patent Specification EP 3 333 256 B1, published October 25, 2023. Title: Method for Producing High-quality iPSCs. Applicant: Heartseed Inc. The sequence listing filed with the application follows.

SEQUENCE LISTING (60 sequences)

SEQ ID NO: 1 - DNA, 624 bp, Homo sapiens
  misc_feature: Inventor:YUASA, Shinsuke; FUKUDA, Keiichi; KUNITOMI, Akira
atggcccccgcgacggctcccaggagagcgggtgaggccaaggggaagggccccaagaaaccaagtgaggccaaggaggaccctcccaacgtgggcaaggtgaaaaaggcagccaagaggccagcaaaggtgcagaagcctcctcccaagccaggcgcagccacagagaaggctcgcaagcaaggcggcgcggccaaggacaccagggcacagtcgggagaggctaggaaggtgccccccaagccagacaaggccatgcgggcaccttccagtgctggtgggctcagcaggaaggcaaaggccaaaggcagcaggagcagccaaggagatgctgaggcctacaggaaaaccaaagctgagagtaagagttcaaaacccacggccagcaaggtcaagaatggtgctgcttccccgaccaaaaagaaggtggtggccaaggccaaggcccctaaagctgggcaggggccaaacaccaaggctgctgctcctgctaagggcagtgggtccaaggtggtacctgcacatttgtccaggaagacagaggcccccaagggccctagaaaggctgggctgcccatcaaggcctcatcatccaaagtgtccagccagagggctgaagcttag

SEQ ID NO: 2 - protein, 207 aa, Homo sapiens
MAPATAPRRAGEAKGKGPKKPSEAKEDPPNVGKVKKAAKRPAKVQKPPPKPGAATEKARKQGGAAKDTRAQSGEARKVPPKPDKAMRAPSSAGGLSRKAKAKGSRSSQGDAEAYRKTKAESKSSKPTASKVKNGAASPTKKKVVAKAKAPKAGQGPNTKAAAPAKGSGSKVVPAHLSRKTEAPKGPRKAGLPIKASSSKVSSQRAEA

SEQ ID NO: 3 - DNA, 915 bp, Mus musculus
atggctcctgggagtgtctccagtgtttcttcctcctcttttccctccagggacacatccccttctggatcatgtgggctccctggagctgacaagccaggtccaagttgccgcagaatccaagcaggccaaaggaacccaacaatgctgcacatggtgctagaggctttgaaggcccgggaggcacgccagggcacatcagttgtagccatcaaggtctacatccaacacaagtacccgacagtggacaccacccgtttcaagtacctgttgaagcaagctctggaaactggcgttcgtcgaggcctcctcaccaggcctgctcactccaaggccaagggtgccactggcagcttcaaactagttccaaagcccaagacaaagaaagcctgtgcccccaaagccggcaggggagctgcaggtgccaaggagacaggctccaagaaatctggattgctgaagaaagaccaagttggcaaggccacgatggagaaagggcagaagaggagggcttacccttgcaaggcagccacactggagatggcacctaagaaagccaaggcgaaaccgaaagaggtcagaaaggctcccctaaaacaagacaaagcagcaggggcccctctgactgccaatggaggccagaaggtcaaacgcagtgggagcaggcaagaagcaaatgcccatgggaaaaccaaaggtgagaaatcgaagcccttggccagcaaggtccagaatagcgttgcttccctcgccaaaaggaagatggcagacatggcccacactgtgacagttgttcagggggctgagacagtacaggagaccaaagtgcccactccttcccaggacataggacacaaagtacaacccatacctagggtcaggaaggcaaagacccctgagaacactcaggcctga

SEQ ID NO: 4 - protein, 304 aa, Mus musculus
MAPGSVSSVSSSSFPSRDTSPSGSCGLPGADKPGPSCRRIQAGQRNPTMLHMVLEALKAREARQGTSVVAIKVYIQHKYPTVDTTRFKYLLKQALETGVRRGLLTRPAHSKAKGATGSFKLVPKPKTKKACAPKAGRGAAGAKETGSKKSGLLKKDQVGKATMEKGQKRRAYPCKAATLEMAPKKAKAKPKEVRKAPLKQDKAAGAPLTANGGQKVKRSGSRQEANAHGKTKGEKSKPLASKVQNSVASLAKRKMADMAHTVTVVQGAETVQETKVPTPSQDIGHKVQPIPRVRKAKTPENTQA

SEQ ID NO: 5 - DNA, 21 bp, Artificial
  Nanog-F
agggtctgctactgagatgct

SEQ ID NO: 6 - DNA, 24 bp, Artificial
  Nanog-R
caacacctggtttttctgccaccg

SEQ ID NO: 7 - DNA, 23 bp, Artificial
  endogenous Oct3/4-F
tctttccaccaggcccccggctc

SEQ ID NO: 8 - DNA, 23 bp, Artificial
  endogenous Oct3/4-R
tgcgggcggacatggggagatcc

SEQ ID NO: 9 - DNA, 23 bp, Artificial
  endogenous Sox2-F
tagagatagactccgggcgatga

SEQ ID NO: 10 - DNA, 23 bp, Artificial
  endogenous Sox2-R
ttgccttaaacaagaccacgaaa

SEQ ID NO: 11 - DNA, 23 bp, Artificial
  exogenous Oct3/4-F
ccccagggccccattttggtacc

SEQ ID NO: 12 - DNA, 23 bp, Artificial
  exogenous Oct3/4-R
ccctttttctggagactaataaa

SEQ ID NO: 13 - DNA, 26 bp, Artificial
  exogenous Sox2-F
ggcacccctggcatggctcttggctc

SEQ ID NO: 14 - DNA, 24 bp, Artificial
  exogenous Sox2-R
ttatcgtcgaccactgtgctgctg

SEQ ID NO: 15 - DNA, 24 bp, Artificial
  Rex1-F
acgagtggcagtttcttcttggga

SEQ ID NO: 16 - DNA, 24 bp, Artificial
  Rex1-R
tatgactcacttccagggggcact

SEQ ID NO: 17 - DNA, 20 bp, Artificial
  Sall4-F
ccctgggaactgcgatgaag

SEQ ID NO: 18 - DNA, 23 bp, Artificial
  Sall4-R
tcagagagactaaagaactcggc

SEQ ID NO: 19 - DNA, 20 bp, Artificial
  H1foo-F
ggcacaggctttctttgtct

SEQ ID NO: 20 - DNA, 20 bp, Artificial
  H1foo-R
tccaacacaagtacccgaca

SEQ ID NO: 21 - DNA, 20 bp, Artificial
  Foxa2-F
agcaccattacgccttcaac

SEQ ID NO: 22 - DNA, 20 bp, Artificial
  Foxa2-R
ccttgaggtccattttgtgg

SEQ ID NO: 23 - DNA, 20 bp, Artificial
  Cxcr4-F
cgggatgaaaacgtccattt

SEQ ID NO: 24 - DNA, 21 bp, Artificial
  Cxcr4-R
atgaccaggatcaccaatcca

SEQ ID NO: 25 - DNA, 22 bp, Artificial
  Col6a2-F
ccaccactgaaaggaacaacaa

SEQ ID NO: 26 - DNA, 23 bp, Artificial
  Col6a2-R
tccaacacgaaatacacgttgac

SEQ ID NO: 27 - DNA, 20 bp, Artificial
  T-F
tgtcctcccttgttgcctta

SEQ ID NO: 28 - DNA, 20 bp, Artificial
  T-R
atgttccaagggcagaacag

SEQ ID NO: 29 - DNA, 20 bp, Artificial
  beta3-Tubulin-F
cccagcggcaactatgtagg

SEQ ID NO: 30 - DNA, 19 bp, Artificial
  beta3-Tubulin-R
ccagaccgaacactgtcca

SEQ ID NO: 31 - DNA, 20 bp, Artificial
  Tubb3-F
ccaaatctacccaccaagga

SEQ ID NO: 32 - DNA, 20 bp, Artificial
  Tubb3-R
agagcttccagaacgtcgag

SEQ ID NO: 33 - DNA, 20 bp, Artificial
  Ki67-F
tctgatgttaggtgtttgag

SEQ ID NO: 34 - DNA, 21 bp, Artificial
  Ki67-R
cacttttctggtaacttcttg

SEQ ID NO: 35 - DNA, 20 bp, Artificial
  PCNA-F
taaagaagaggaggcggtaa

SEQ ID NO: 36 - DNA, 20 bp, Artificial
  PCNA-R
taagtgtcccatgtcagcaa

SEQ ID NO: 37 - DNA, 19 bp, Artificial
  GAPDH-F
ttcaacggcacagtcaagg

SEQ ID NO: 38 - DNA, 19 bp, Artificial
  GAPDH-R
catggactgtggtcatgag

SEQ ID NO: 39 - DNA, 24 bp, Artificial
  Oct3/4-DMR-F
ggttttttagaggatggttgagtg

SEQ ID NO: 40 - DNA, 23 bp, Artificial
  Oct3/4-DMR-R
tccaaccctactaacccatcacc

SEQ ID NO: 41 - DNA, 30 bp, Artificial
  Nanog-DMR-F
gattttgtaggtgggattaattgtgaattt

SEQ ID NO: 42 - DNA, 30 bp, Artificial
  Nanog-DMR-R
accaaaaaaacccacactcatatcaatata

SEQ ID NO: 43 - DNA, 22 bp, Artificial
  IG-DMR-F
gtggtttgttatgggtaagttt

SEQ ID NO: 44 - DNA, 24 bp, Artificial
  IG-DMR-R
cccttccctcactccaaaaattaa

SEQ ID NO: 45 - DNA, 28 bp, Artificial
  Gtl2-DMR-F
agttattttttgtttgaaaggatgtgta

SEQ ID NO: 46 - DNA, 28 bp, Artificial
  Gtl2-DMR-R
ctaactttaaaaaaaaatccccaacact

SEQ ID NO: 47 - DNA, 1083 bp, Homo sapiens
atggcgggacacctggcttcggatttcgccttctcgccccctccaggtggtggaggtgatgggccaggggggccggagccgggctgggttgatcctcggacctggctaagcttccaaggccctcctggagggccaggaatcgggccgggggttgggccaggctctgaggtgtgggggattcccccatgccccccgccgtatgagttctgtggggggatggcgtactgtgggccccaggttggagtggggctagtgccccaaggcggcttggagacctctcagcctgagggcgaagcaggagtcggggtggagagcaactccgatggggcctccccggagccctgcaccgtcacccctggtgccgtgaagctggagaaggagaagctggagcaaaacccggaggagtcccaggacatcaaagctctgcagaaagaactcgagcaatttgccaagctcctgaagcagaagaggatcaccctgggatatacacaggccgatgtggggctcaccctgggggttctatttgggaaggtattcagccaaacgaccatctgccgctttgaggctctgcagcttagcttcaagaacatgtgtaagctgcggcccttgctgcagaagtgggtggaggaagctgacaacaatgaaaatcttcaggagatatgcaaagcagaaaccctcgtgcaggcccgaaagagaaagcgaaccagtatcgagaaccgagtgagaggcaacctggagaatttgttcctgcagtgcccgaaacccacactgcagcagatcagccacatcgcccagcagcttgggctcgagaaggatgtggtccgagtgtggttctgtaaccggcgccagaagggcaagcgatcaagcagcgactatgcacaacgagaggattttgaggctgctgggtctcctttctcagggggaccagtgtcctttcctctggccccagggccccattttggtaccccaggctatgggagccctcacttcactgcactgtactcctcggtccctttccctgagggggaagcctttccccctgtctccgtcaccactctgggctctcccatgcattcaaactga

SEQ ID NO: 48 - protein, 360 aa, Homo sapiens
MAGHLASDFAFSPPPGGGGDGPGGPEPGWVDPRTWLSFQGPPGGPGIGPGVGPGSEVWGIPPCPPPYEFCGGMAYCGPQVGVGLVPQGGLETSQPEGEAGVGVESNSDGASPEPCTVTPGAVKLEKEKLEQNPEESQDIKALQKELEQFAKLLKQKRITLGYTQADVGLTLGVLFGKVFSQTTICRFEALQLSFKNMCKLRPLLQKWVEEADNNENLQEICKAETLVQARKRKRTSIENRVRGNLENLFLQCPKPTLQQISHIAQQLGLEKDVVRVWFCNRRQKGKRSSSDYAQREDFEAAGSPFSGGPVSFPLAPGPHFGTPGYGSPHFTALYSSVPFPEGEAFPPVSVTTLGSPMHSN

SEQ ID NO: 49 - DNA, 954 bp, Homo sapiens
atgtacaacatgatggagacggagctgaagccgccgggcccgcagcaaacttcggggggcggcggcggcaactccaccgcggcggcggccggcggcaaccagaaaaacagcccggaccgcgtcaagcggcccatgaatgccttcatggtgtggtcccgcgggcagcggcgcaagatggcccaggagaaccccaagatgcacaactcggagatcagcaagcgcctgggcgccgagtggaaacttttgtcggagacggagaagcggccgttcatcgacgaggctaagcggctgcgagcgctgcacatgaaggagcacccggattataaataccggccccggcggaaaaccaagacgctcatgaagaaggataagtacacgctgcccggcgggctgctggcccccggcggcaatagcatggcgagcggggtcggggtgggcgccggcctgggcgcgggcgtgaaccagcgcatggacagttacgcgcacatgaacggctggagcaacggcagctacagcatgatgcaggaccagctgggctacccgcagcacccgggcctcaatgcgcacggcgcagcgcagatgcagcccatgcaccgctacgacgtgagcgccctgcagtacaactccatgaccagctcgcagacctacatgaacggctcgcccacctacagcatgtcctactcgcagcagggcacccctggcatggctcttggctccatgggttcggtggtcaagtccgaggccagctccagcccccctgtggttacctcttcctcccactccagggcgccctgccaggccggggacctccgggacatgatcagcatgtatctccccggcgccgaggtgccggaacccgccgcccccagcagacttcacatgtcccagcactaccagagcggcccggtgcccggcacggccattaacggcacactgcccctctcacacatgtga

SEQ ID NO: 50 - protein, 317 aa, Homo sapiens
MYNMMETELKPPGPQQTSGGGGGNSTAAAAGGNQKNSPDRVKRPMNAFMVWSRGQRRKMAQENPKMHNSEISKRLGAEWKLLSETEKRPFIDEAKRLRALHMKEHPDYKYRPRRKTKTLMKKDKYTLPGGLLAPGGNSMASGVGVGAGLGAGVNQRMDSYAHMNGWSNGSYSMMQDQLGYPQHPGLNAHGAAQMQPMHRYDVSALQYNSMTSSQTYMNGSPTYSMSYSQQGTPGMALGSMGSVVKSEASSSPPVVTSSSHSRAPCQAGDLRDMISMYLPGAEVPEPAAPSRLHMSQHYQSGPVPGTAINGTLPLSHM

SEQ ID NO: 51 - DNA, 1440 bp, Homo sapiens
atgaggcagccacctggcgagtctgacatggctgtcagcgacgcgctgctcccatctttctccacgttcgcgtctggcccggcgggaagggagaagacactgcgtcaagcaggtgccccgaataaccgctggcgggaggagctctcccacatgaagcgacttcccccagtgcttcccggccgcccctatgacctggcggcggcgaccgtggccacagacctggagagcggcggagccggtgcggcttgcggcggtagcaacctggcgcccctacctcggagagagaccgaggagttcaacgatctcctggacctggactttattctctccaattcgctgacccatcctccggagtcagtggccgccaccgtgtcctcgtcagcgtcagcctcctcttcgtcgtcgccgtcgagcagcggccctgccagcgcgccctccacctgcagcttcacctatccgatccgggccgggaacgacccgggcgtggcgccgggcggcacgggcggaggcctcctctatggcagggagtccgctccccctccgacggctcccttcaacctggcggacatcaacgacgtgagcccctcgggcggcttcgtggccgagctcctgcggccagaattggacccggtgtacattccgccgcagcagccgcagccgccaggtggcgggctgatgggcaagttcgtgctgaaggcgtcgctgagcgcccctggcagcgagtacggcagcccgtcggtcatcagcgtcagcaaaggcagccctgacggcagccacccggtggtggtggcgccctacaacggcgggccgccgcgcacgtgccccaagatcaagcaggaggcggtctcttcgtgcacccacttgggcgctggaccccctctcagcaatggccaccggccggctgcacacgacttccccctggggcggcagctccccagcaggactaccccgaccctgggtcttgaggaagtgctgagcagcagggactgtcaccctgccctgccgcttcctcccggcttccatccccacccggggcccaattacccatccttcctgcccgatcagatgcagccgcaagtcccgccgctccattaccaagagctcatgccacccggttcctgcatgccagaggagcccaagccaaagaggggaagacgatcgtggccccggaaaaggaccgccacccacacttgtgattacgcgggctgcggcaaaacctacacaaagagttcccatctcaaggcacacctgcgaacccacacaggtgagaaaccttaccactgtgactgggacggctgtggatggaaattcgcccgctcagatgaactgaccaggcactaccgtaaacacacggggcaccgcccgttccagtgccaaaaatgcgaccgagcattttccaggtcggaccacctcgccttacacatgaagaggcatttttaa

SEQ ID NO: 52 - protein, 479 aa, Homo sapiens
MRQPPGESDMAVSDALLPSFSTFASGPAGREKTLRQAGAPNNRWREELSHMKRLPPVLPGRPYDLAAATVATDLESGGAGAACGGSNLAPLPRRETEEFNDLLDLDFILSNSLTHPPESVAATVSSSASASSSSSPSSSGPASAPSTCSFTYPIRAGNDPGVAPGGTGGGLLYGRESAPPPTAPFNLADINDVSPSGGFVAELLRPELDPVYIPPQQPQPPGGGLMGKFVLKASLSAPGSEYGSPSVISVSKGSPDGSHPVVVAPYNGGPPRTCPKIKQEAVSSCTHLGAGPPLSNGHRPAAHDFPLGRQLPSRTTPTLGLEEVLSSRDCHPALPLPPGFHPHPGPNYPSFLPDQMQPQVPPLHYQELMPPGSCMPEEPKPKRGRRSWPRKRTATHTCDYAGCGKTYTKSSHLKAHLRTHTGEKPYHCDWDGCGWKFARSDELTRHYRKHTGHRPFQCQKCDRAFSRSDHLALHMKRHF

SEQ ID NO: 53 - DNA, 1095 bp, Homo sapiens
atggactacgactcgtaccagcactatttctacgactatgactgcggggaggatttctaccgctccacggcgcccagcgaggacatctggaagaaattcgagctggtgccatcgccccccacgtcgccgccctggggcttgggtcccggcgcaggggacccggcccccgggattggtcccccggagccgtggcccggagggtgcaccggagacgaagcggaatcccggggccactcgaaaggctggggcaggaactacgcctccatcatacgccgtgactgcatgtggagcggcttctcggcccgggaacggctggagagagctgtgagcgaccggctcgctcctggcgcgccccgggggaacccgcccaaggcgtccgccgccccggactgcactcccagcctcgaagccggcaacccggcgcccgccgccccctgtccgctgggcgaacccaagacccaggcctgctccgggtccgagagcccaagcgactcggagaatgaagaaattgatgttgtgacagtagagaagaggcagtctctgggtattcggaagccggtcaccatcacggtgcgagcagaccccctggatccctgcatgaagcatttccacatctccatccatcagcaacagcacaactatgctgcccgttttcctccagaaagctgctcccaagaagaggcttcagagaggggtccccaagaagaggttctggagagagatgctgcaggggaaaaggaagatgaggaggatgaagagattgtgagtcccccacctgtagaaagtgaggctgcccagtcctgccaccccaaacctgtcagttctgatactgaggatgtgaccaagaggaagaatcacaacttcctggagcgcaagaggcggaatgacctgcgttcgcgattcttggcgctgagggaccaggtgcccaccctggccagctgctccaaggcccccaaagtagtgatcctaagcaaggccttggaatacttgcaagccctggtgggggctgagaagaggatggctacagagaaaagacagctccgatgccggcagcagcagttgcagaaaagaattgcatacctcactggctactaa

SEQ ID NO: 54 - protein, 364 aa, Homo sapiens
MDYDSYQHYFYDYDCGEDFYRSTAPSEDIWKKFELVPSPPTSPPWGLGPGAGDPAPGIGPPEPWPGGCTGDEAESRGHSKGWGRNYASIIRRDCMWSGFSARERLERAVSDRLAPGAPRGNPPKASAAPDCTPSLEAGNPAPAAPCPLGEPKTQACSGSESPSDSENEEIDVVTVEKRQSLGIRKPVTITVRADPLDPCMKHFHISIHQQQHNYAARFPPESCSQEEASERGPQEEVLERDAAGEKEDEEDEEIVSPPPVESEAAQSCHPKPVSSDTEDVTKRKNHNFLERKRRNDLRSRFLALRDQVPTLASCSKAPKVVILSKALEYLQALVGAEKRMATEKRQLRCRQQQLQKRIAYLTGY

SEQ ID NO: 55 - DNA, 20 bp, Artificial
  SRF-F
acccataagccccagctatc

SEQ ID NO: 56 - DNA, 20 bp, Artificial
  SRF-R
ggtgccaagatggaagtcac

SEQ ID NO: 57 - DNA, 20 bp, Artificial
  ACTG2-F
cggtggtctcctcttcacac

SEQ ID NO: 58 - DNA, 22 bp, Artificial
  ACTG2-R
cactgggagaagaacctctcat

SEQ ID NO: 59 - DNA, 1041 bp, Homo sapiens
atggctcctgggagcgtcaccagcgacatctcaccctcctcgacttccacagcaggatcatccaggtctcctgaatctgaaaagccaggcccgagccacggcggtgtcccaccaggaggcccgagccacagcagcctcccggtgggacgccgccaccccccggtgctacgcatggtgctggaggcgctgcaggctggggagcagcgccggggcacgtcggtggcagctatcaagctctacatcctgcacaagtacccaacagtggacgtcctccgcttcaagtacctgctgaagcaggcgctggccactggcatgcgccgtggcctcctcgccaggcccctcaactccaaagccaggggggccactggcagcttcaaattagttcccaagcacaagaagaaaatccagcccaggaagatggcccccgcgacggctcccaggagagcgggtgaggccaaggggaagggccccaagaaaccaagtgaggccaaggaggaccctcccaacgtgggcaaggtgaaaaaggcagccaagaggccagcaaaggtgcagaagcctcctcccaagccaggcgcagccacagagaaggctcgcaagcaaggcggcgcggccaaggacaccagggcacagtcgggagaggctaggaaggtgccccccaagccagacaaggccatgcgggcaccttccagtgctggtgggctcagcaggaaggcaaaggccaaaggcagcaggagcagccaaggagatgctgaggcctacaggaaaaccaaagctgagagtaagagttcaaaacccacggccagcaaggtcaagaatggtgctgcttccccgaccaaaaagaaggtggtggccaaggccaaggcccctaaagctgggcaggggccaaacaccaaggctgctgctcctgctaagggcagtgggtccaaggtggtacctgcacatttgtccaggaagacagaggcccccaagggccctagaaaggctgggctgcccatcaaggcctcatcatccaaagtgtccagccagagggctgaagcttag

SEQ ID NO: 60 - protein, 346 aa, Homo sapiens
MAPGSVTSDISPSSTSTAGSSRSPESEKPGPSHGGVPPGGPSHSSLPVGRRHPPVLRMVLEALQAGEQRRGTSVAAIKLYILHKYPTVDVLRFKYLLKQALATGMRRGLLARPLNSKARGATGSFKLVPKHKKKIQPRKMAPATAPRRAGEAKGKGPKKPSEAKEDPPNVGKVKKAAKRPAKVQKPPPKPGAATEKARKQGGAAKDTRAQSGEARKVPPKPDKAMRAPSSAGGLSRKAKAKGSRSSQGDAEAYRKTKAESKSSKPTASKVKNGAASPTKKKVVAKAKAPKAGQGPNTKAAAPAKGSGSKVVPAHLSRKTEAPKGPRKAGLPIKASSSKVSSQRAEA